European Patent Specification EP 3 662 287 B1, published February 28, 2024. Title: SYSTEMS AND METHODS FOR PERFORMING A REAL-TIME ASSAY OF A SAMPLE. Applicant: AMGEN INC. Wu, Chao-Hsiang. The sequence listing filed with the application follows.

SEQUENCE LISTING (86 sequences)

SEQ ID NO: 1 - protein, 239 aa, Homo sapiens
MRLPAQLLGLLMLWVPGSSGDIVMTQTPLSSPVTLGQPASISCRSSQSLVHSDGNTYLNWLQQRPGQPPRLLIYKISNRFSGVPDRFTGSGAGTDFTLKISRVEAEDVGVYTCMQVTQFPLTFGQGTRLEIKRTVAAPSVFIFPPSDEQLKSGTASVVCLLNNFYPREAKVQWKVDNALQSGNSQESVTEQDSKDSTYSLSSTLTLSKADYEKHKVYACEVTHQGLSSPVTKSFNRGEC

SEQ ID NO: 2 - protein, 470 aa, Homo sapiens [sequence omitted]

SEQ ID NO: 3 - protein, 235 aa, Homo sapiens
METPAQLLFLLLLWLPDTTGEIVLTQSPGTLSLSPGDRATLSCRASQSVSSSYFAWYQQKPGQAPRLLIYGASSRATGIPDRFSGSGSGTDFTLTISRLEPEDFAVYYCQQYDRSPRTFGQGTKVEIKRTVAAPSVFIFPPSDEQLKSGTASVVCLLNNFYPREAKVQWKVDNALQSGNSQESVTEQDSKDSTYSLSSTLTLSKADYEKHKVYACEVTHQGLSSPVTKSFNRGEC

SEQ ID NO: 4 - protein, 463 aa, Homo sapiens
MDWTWRILFLVAAATGAHSQVQLVQSGAEVKKPGASVKVSCKSSGYTFTGYYMHWVRQAPGQGLEWMGWINPNSGGTNYAQKFKGRVTMTRDTSISTAYMELSRLRSDDTAVYYCARDKWLDGFDYWGQGTLVTVSSASTKGPSVFPLAPCSRSTSESTAALGCLVKDYFPEPVTVSWNSGALTSGVHTFPAVLQSSGLYSLSSVVTVPSSNFGTQTYTCNVDHKPSNTKVDKTVERKCCVECPPCPAPPVAGPSVFLFPPKPKDTLMISRTPEVTCVVVDVSHEDPEVQFNWYVDGVEVHNAKTKPREEQFNSTFRVVSVLTVVHQDWLNGKEYKCKVSNKGLPAPIEKTISKTKGQPREPQVYTLPPSREEMTKNQVSLTCLVKGFYPSDIAVEWESNGQPENNYKTTPPMLDSDGSFFLYSKLTVDKSRWQQGNVFSCSVMHEALHNHYTQKSLSLSPGK

SEQ ID NO: 5 - protein, 235 aa, Homo sapiens
MAWALLLLTLLTQDTGSWAQSVLTQSPSASGTPGQRVTISCSGSSSNIGSNYVYWYQQLPGAAPKLLILRNNQRPSGVPDRFSGSKSGTSASLTISGLRSEDEADYYCAAWDDSLSGWVFGGGTKLTVLGQPKANPTVTLFPPSSEELQANKATLVCLISDFYPGAVTVAWKADGSPVKAGVETTKPSKQSNNKYAASSYLSLTPEQWKSHRSYSCQVTHEGSTVEKTVAPTECS

SEQ ID NO: 6 - protein, 479 aa, Homo sapiens
MDMRVPAQLLGLLLLWLRGARCEVQLVESGGGLVKPGGSLRLSCAASGFTFSNAWMSWVRQAPGKGLEWVGRIKSKTDGGTTDYTAPVKGRFTISRDDSKNTLYLQMNSLKAEDTAVYYCTTDRTGYSISWSSYYYYYGMDVWGQGTTVTVSSASTKGPSVFPLAPCSRSTSESTAALGCLVKDYFPEPVTVSWNSGALTSGVHTFPAVLQSSGLYSLSSVVTVPSSNFGTQTYTCNVDHKPSNTKVDKTVERKCCVECPPCPAPPVAGPSVFLFPPKPKDTLMISRTPEVTCVVVDVSHEDPEVQFNWYVDGVEVHNAKTKPREEQFNSTFRVVSVLTVVHQDWLNGKEYKCKVSNKGLPAPIEKTISKTKGQPREPQVYTLPPSREEMTKNQVSLTCLVKGFYPSDIAVEWESNGQPENNYKTTPPMLDSDGSFFLYSKLTVDKSRWQQGNVFSCSVMHEALHNHYTQKSLSLSPGK

SEQ ID NO: 7 - protein, 235 aa, Homo sapiens
METPAQLLFLLLLWLPDTTGEIVLTQSPGTLSLSPGERATLSCRASQSVRGRYLAWYQQKPGQAPRLLIYGASSRATGIPDRFSGSGSGTDFTLTISRLEPEDFAVFYCQQYGSSPRTFGQGTKVEIKRTVAAPSVFIFPPSDEQLKSGTASVVCLLNNFYPREAKVQWKVDNALQSGNSQESVTEQDSKDSTYSLSSTLTLSKADYEKHKVYACEVTHQGLSSPVTKSFNRGEC

SEQ ID NO: 8 - protein, 467 aa, Homo sapiens
MEFGLSWLFLVAILKGVQCEVQLLESGGGLVQPGGSLRLSCAASGFTFSSYAMSWVRQAPGKGLEWVSGITGSGGSTYYADSVKGRFTISRDNSKNTLYLQMNSLRAEDTAVYYCAKDPGTTVIMSWFDPWGQGTLVTVSSASTKGPSVFPLAPCSRSTSESTAALGCLVKDYFPEPVTVSWNSGALTSGVHTFPAVLQSSGLYSLSSVVTVPSSNFGTQTYTCNVDHKPSNTKVDKTVERKCCVECPPCPAPPVAGPSVFLFPPKPKDTLMISRTPEVTCVVVDVSHEDPEVQFNWYVDGVEVHNAKTKPREEQFNSTFRVVSVLTVVHQDWLNGKEYKCKVSNKGLPAPIEKTISKTKGQPREPQVYTLPPSREEMTKNQVSLTCLVKGFYPSDIAVEWESNGQPENNYKTTPPMLDSDGSFFLYSKLTVDKSRWQQGNVFSCSVMHEALHNHYTQKSLSLSPGK

SEQ ID NO: 9 - protein, 242 aa, Homo sapiens
MDMRVPAQLLGLLLLWLRGARCDIVMTQTPLSLPVTPGEPASISCRSSQSLLNSVDGSTNLDWYLQKPGQSPQLLIYTLSYRASGVPDRFSGSGSGTDFTLKISRVEAEDVGVYYCMQRIEFPLTFGGGTKVEIKRTVAAPSVFIFPPSDEQLKSGTASVVCLLNNFYPREAKVQWKVDNALQSGNSQESVTEQDSKDSTYSLSSTLTLSKADYEKHKVYACEVTHQGLSSPVTKSFNRGEC

SEQ ID NO: 10 - protein, 465 aa, Homo sapiens
MELGLCWVFLVAILEGVQCEVQLVESGGGLVQPGGSLRLSCAASGFTFSSYSMNWVRQAPGKGLEWVSYISSSGSSIYYADSVKGRFTISRDNAKNSLYLQMNSLRDEDTAVYYCARERYYGDTPFDYWGQGTLVTVSSASTKGPSVFPLAPCSRSTSESTAALGCLVKDYFPEPVTVSWNSGALTSGVHTFPAVLQSSGLYSLSSVVTVPSSNFGTQTYTCNVDHKPSNTKVDKTVERKCCVECPPCPAPPVAGPSVFLFPPKPKDTLMISRTPEVTCVVVDVSHEDPEVQFNWYVDGVEVHNAKTKPREEQFNSTFRVVSVLTVVHQDWLNGKEYKCKVSNKGLPAPIEKTISKTKGQPREPQVYTLPPSREEMTKNQVSLTCLVKGFYPSDIAVEWESNGQPENNYKTTPPMLDSDGSFFLYSKLTVDKSRWQQGNVFSCSVMHEALHNHYTQKSLSLSPGK

SEQ ID NO: 11 - protein, 233 aa, Homo sapiens
MSPSQLIGFLLLWVPASRGEIVLTQSPDFQSVTPKEKVTITCRASQSIGSSLHWYQQKPDQSPKLLIKYASQSFSGVPSRFSGSGSGTDFTLTINSLEAEDAAAYYCHQSSSLPLTFGGGTKVEIKRTVAAPSVFIFPPSDEQLKSGTASVVCLLNNFYPREAKVQWKVDNALQSGNSQESVTEQDSKDSTYSLSSTLTLSKADYEKHKVYACEVTHQGLSSPVTKSFNRGEC

SEQ ID NO: 12 - protein, 463 aa, Homo sapiens
MGSTAILALLLAVLQGVCAEVQLMQSGAEVKKPGESLKISCKGSGYSFSFHWIAWVRQMPGKGLEWMGIIHPGASDTRYSPSFQGQVTISADNSNSATYLQWSSLKASDTAMYFCARQRELDYFDYWGQGTLVTVSSASTKGPSVFPLAPCSRSTSESTAALGCLVKDYFPEPVTVSWNSGALTSGVHTFPAVLQSSGLYSLSSVVTVPSSNFGTQTYTCNVDHKPSNTKVDKTVERKCCVECPPCPAPPVAGPSVFLFPPKPKDTLMISRTPEVTCVVVDVSHEDPEVQFNWYVDGVEVHNAKTKPREEQFNSTFRVVSVLTVVHQDWLNGKEYKCKVSNKGLPAPIEKTISKTKGQPREPQVYTLPPSREEMTKNQVSLTCLVKGFYPSDIAVEWESNGQPENNYKTTPPMLDSDGSFFLYSKLTVDKSRWQQGNVFSCSVMHEALHNHYTQKSLSLSPGK

SEQ ID NO: 13 - protein, 236 aa, Homo sapiens
MDMRVPAQLLGLLLLWLRGARCDIQMTQSPSSLSASVGDRVTITCKASQDINKYVAWYQQKPGKAPKLLIYYTSWLQPGVPSRFSGSGSGTDFTFTISSLQPEDIATYYCLQYDNLLYTFGQGTKLEIKRTVAAPSVFIFPPSDEQLKSGTASVVCLLNNFYPREAKVQWKVDNALQSGNSQESVTEQDSKDSTYSLSSTLTLSKADYEKHKVYACEVTHQGLSSPVTKSFNRGEC

SEQ ID NO: 14 - protein, 467 aa, Homo sapiens
MDMRVPAQLLGLLLLWLRGARCEVQLVESGGGLVQPGGSLRLSCAASGFTFSRYWMNWVRQAPGKGLEWVAQIRLKSDNYATHYAESVKGRFTISRDNAKNSLYLQMNSLRAEDTAVYYCTEGLDYWGQGTTVTVSSASTKGPSVFPLAPSSKSTSGGTAALGCLVKDYFPEPVTVSWNSGALTSGVHTFPAVLQSSGLYSLSSVVTVPSSSLGTQTYICNVNHKPSNTKVDKKVEPKSCDKTHTCPPCPAPELLGGPSVFLFPPKPKDTLMISRTPEVTCVVVDVSHEDPEVKFNWYVDGVEVHNAKTKPREEQYNSTYRVVSVLTVLHQDWLNGKEYKCKVSNKALPAPIEKTISKAKGQPREPQVYTLPPSREEMTKNQVSLTCLVKGFYPSDIAVEWESNGQPENNYKTTPPVLDSDGSFFLYSKLTVDKSRWQQGNVFSCSVMHEALHNHYTQKSLSLSPGK

SEQ ID NO: 15 - protein, 236 aa, Homo sapiens
MDMRVLAQLLGLLLLCFPGARCDIQMTQSPSSLSASVGDRVTITCRASQGISNWLAWYQQKPEKAPKSLIYAASSLQSGVPSRFSGSGSGTDFTLTISSLQPEDFATYYCQQYDSYPRTFGQGTKVEIKRTVAAPSVFIFPPSDEQLKSGTASVVCLLNNFYPREAKVQWKVDNALQSGNSQESVTEQDSKDSTYSLSSTLTLSKADYEKHKVYACEVTHQGLSSPVTKSFNRGEC

SEQ ID NO: 16 - protein, 466 aa, Homo sapiens
MELGLNWVFLVAILEGVHCEVQLVESGGGLVQPGGSLRLSCAASGFTFSSYWMSWVRQAPGKGLEWVAYIKQDGNEKYYVDSVKGRFTISRDNAKNSLYLQMNSLRAEDTAVYYCAREGILWFGDLPTFWGQGTLVTVSSASTKGPSVFPLAPCSRSTSESTAALGCLVKDYFPEPVTVSWNSGALTSGVHTFPAVLQSSGLYSLSSVVTVPSSNFGTQTYTCNVDHKPSNTKVDKTVERKCCVECPPCPAPPVAGPSVFLFPPKPKDTLMISRTPEVTCVVVDVSHEDPEVQFNWYVDGVEVHNAKTKPREEQFNSTFRVVSVLTVVHQDWLNGKEYKCKVSNKGLPAPIEKTISKTKGQPREPQVYTLPPSREEMTKNQVSLTCLVKGFYPSDIAVEWESNGQPENNYKTTPPMLDSDGSFFLYSKLTVDKSRWQQGNVFSCSVMHEALHNHYTQKSLSLSPGK

SEQ ID NO: 17 - protein, 241 aa, Homo sapiens
MDMRLPAQLLGLLMLWVPGSSGDVLMTQSPLSLPVTLGQPASISCRSSQSIVHSNGNTYLEWYLQRPGQSPKLLIYKVSNRFSGVPDRFSGSGSGTDFTLKISRVEAEDVGVYYCFQGSHVPLTFGAGTKLEIKRTVAAPSVFIFPPSDEQLKSGTASVVCLLNNFYPREAKVQWKVDNALQSGNSQESVTEQDSKDSTYSLSSTLTLSKADYEKHKVYACEVTHQGLSSPVTKSFNRGEC

SEQ ID NO: 18 - protein, 470 aa, Homo sapiens
MDTLCSTLLLLTIPSWVLSQVTLKESGPALVKPTQTLTLTCTFSGFSLRTSGMGVGWIRQPPGKALEWLAHIWWDDDKSYNPSLKSQLTISKDTSKNQVVLTMTNMDPVDTATYYCARRNYYYDDYFAYWGQGTLVTVSSASTKGPSVFPLAPSSKSTSGGTAALGCLVKDYFPEPVTVSWNSGALTSGVHTFPAVLQSSGLYSLSSVVTVPSSSLGTQTYICNVNHKPSNTKVDKKVEPKSCDKTHTCPPCPAPELLGGPSVFLFPPKPKDTLMISRTPEVTCVVVDVSHEDPEVKFNWYVDGVEVHNAKTKPREEQYNSTYRVVSVLTVLHQDWLNGKEYKCKVSNKALPAPIEKTISKAKGQPREPQVYTLPPSRDELTKNQVSLTCLVKGFYPSDIAVEWESNGQPENNYKTTPPVLDSDGSFFLYSKLTVDKSRWQQGNVFSCSVMHEALHNHYTQKSLSLSPGK

SEQ ID NO: 19 - protein, 235 aa, Homo sapiens
METPAQLLFLLLLWLPDTTGEIVLTQSPGTLSLSPGERATLSCRASQSVSSSYFAWYQQKPGQAPRLLIYGTSSRATGIPDRFSGSGSGTDFTLTVSRLEPEDFAVYYCQQYDRSPRTFGQGTKVEIKRTVAAPSVFIFPPSDEQLKSGTASVVCLLNNFYPREAKVQWKVDNALQSGNSQESVTEQDSKDSTYSLSSTLTLSKADYEKHKVYACEVTHQGLSSPVTKSFNRGEC

SEQ ID NO: 20 - protein, 463 aa, Homo sapiens
MDWTWRILFLVAAATGAHSQVQLVQSGAAVKKPGASVKVSCKASGYTFTGYYIHWVRQAPGQGLEWMGWINPNSGGTNYAQKFQGRVTMTRDTSISTASMELSRLRSDDTAVYFCARDRWLDAFDIWGQGTMVTVSSASTKGPSVFPLAPCSRSTSESTAALGCLVKDYFPEPVTVSWNSGALTSGVHTFPAVLQSSGLYSLSSVVTVPSSNFGTQTYTCNVDHKPSNTKVDKTVERKCCVECPPCPAPPVAGPSVFLFPPKPKDTLMISRTPEVTCVVVDVSHEDPEVQFNWYVDGVEVHNAKTKPREEQFNSTFRVVSVLTVVHQDWLNGKEYKCKVSNKGLPAPIEKTISKTKGQPREPQVYTLPPSREEMTKNQVSLTCLVKGFYPSDIAVEWESNGQPENNYKTTPPMLDSDGSFFLYSKLTVDKSRWQQGNVFSCSVMHEALHNHYTQKSLSLSPGK

SEQ ID NO: 21 - protein, 235 aa, Homo sapiens
METPAQLLFLLLLWLPDTTGEIVLTQSPGTLSLSPGERATLSCRASQSVSSGYLTWYQQKPGQAPRLLIYGASSRATGIPDRFSGSGSGTDFTLTISRLEPEDFAVYYCQQYGNSLSRFGQGTKLEIKRTVAAPSVFIFPPSDEQLKSGTASVVCLLNNFYPREAKVQWKVDNALQSGNSQESVTEQDSKDSTYSLSSTLTLSKADYEKHKVYACEVTHQGLSSPVTKSFNRGEC

SEQ ID NO: 22 - protein, 474 aa, Homo sapiens
MDMRVPAQLLGLLLLWLRGARCQVQLVESGGGVVQPGRSLRLSCAASGFTFSSYGMHWVRQAPGKGLEWVAVIWYDGSNKYYADSVKGRFIISRDKSKNTLYLQMNSLRAEDTAVYYCARAGGIAAAGLYYYYGMDVWGQGTTVTVSSASTKGPSVFPLAPCSRSTSESTAALGCLVKDYFPEPVTVSWNSGALTSGVHTFPAVLQSSGLYSLSSVVTVPSSNFGTQTYTCNVDHKPSNTKVDKTVERKCCVECPPCPAPPVAGPSVFLFPPKPKDTLMISRTPEVTCVVVDVSHEDPEVQFNWYVDGVEVHNAKTKPREEQFNSTFRVVSVLTVVHQDWLNGKEYKCKVSNKGLPAPIEKTISKTKGQPREPQVYTLPPSREEMTKNQVSLTCLVKGFYPSDIAVEWESNGQPENNYKTTPPMLDSDGSFFLYSKLTVDKSRWQQGNVFSCSVMHEALHNHYTQKSLSLSPGK

SEQ ID NO: 23 - protein, 236 aa, Homo sapiens
MDMRVPAQLLGLLLLWLRGARCSSELTQDPTVSVALGQTVKITCQGDSLRSFYASWYQQKPGQAPVLVFYGKNNRPSGIPDRFSGSSSGNTASLTITGAQAEDEADYYCNSRDSSVYHLVLGGGTKLTVLGQPKANPTVTLFPPSSEELQANKATLVCLISDFYPGAVTVAWKADGSPVKAGVETTKPSKQSNNKYAASSYLSLTPEQWKSHRSYSCQVTHEGSTVEKTVAPTECS

SEQ ID NO: 24 - protein, 478 aa, Homo sapiens
MDMRVPAQLLGLLLLWLRGARCQVQLVQSGAEVKKPGASVKVSCKASGYTFTGYYMHWVRQAPGQGLEWMGWINPNSGGTNYAQKFQGRVTMTRDTSISTAYMELSRLRSDDTAVYFCARDQMSIIMLRGVFPPYYYGMDVWGQGTTVTVSSASTKGPSVFPLAPCSRSTSESTAALGCLVKDYFPEPVTVSWNSGALTSGVHTFPAVLQSSGLYSLSSVVTVPSSNFGTQTYTCNVDHKPSNTKVDKTVERKCCVECPPCPAPPVAGPSVFLFPPKPKDTLMISRTPEVTCVVVDVSHEDPEVQFNWYVDGVEVHNAKTKPREEQFNSTFRVVSVLTVVHQDWLNGKEYKCKVSNKGLPAPIEKTISKTKGQPREPQVYTLPPSREEMTKNQVSLTCLVKGFYPSDIAVEWESNGQPENNYKTTPPMLDSDGSFFLYSKLTVDKSRWQQGNVFSCSVMHEALHNHYTQKSLSLSPGK

SEQ ID NO: 25 - protein, 241 aa, Homo sapiens
MDMRVPAQLLGLLLLWLRGARCDIVMTQSPLSLPVTPGEPASISCRSSQSLLHSNGYNYLDWYLQKPGQSPQLLIYLGSNRASGVPDRFSGSGSGTDFTLKISRVEAEDVGVYYCMQALQTPLTFGGGTKVEIKRTVAAPSVFIFPPSDEQLKSGTASVVCLLNNFYPREAKVQWKVDNALQSGNSQESVTEQDSKDSTYSLSSTLTLSKADYEKHKVYACEVTHQGLSSPVTKSFNRGEC

SEQ ID NO: 26 - protein, 475 aa, Homo sapiens
MDMRVPAQLLGLLLLWLRGARCEVQLVESGGGLVQPGGSLRLSCAASGFTFSSYWMSWVRQAPGKGLEWVASIKQDGSEKYYVDSVKGRFTISRDNARNSLYLQMNSLRAEDTAVYYCARDLVLMVYDIDYYYYGMDVWGQGTTVTVSSASTKGPSVFPLAPCSRSTSESTAALGCLVKDYFPEPVTVSWNSGALTSGVHTFPAVLQSSGLYSLSSVVTVPSSNFGTQTYTCNVDHKPSNTKVDKTVERKCCVECPPCPAPPVAGPSVFLFPPKPKDTLMISRTPEVTCVVVDVSHEDPEVQFNWYVDGVEVHNAKTKPREEQFNSTFRVVSVLTVVHQDWLNGKEYKCKVSNKGLPAPIEKTISKTKGQPREPQVYTLPPSREEMTKNQVSLTCLVKGFYPSDIAVEWESNGQPENNYKTTPPMLDSDGSFFLYSKLTVDKSRWQQGNVFSCSVMHEALHNHYTQKSLSLSPGK

SEQ ID NO: 27 - protein, 241 aa, Homo sapiens
MDMRVPAQLLGLLLLWLRGARCDIVMTQSPLSLPVTPGEPASISCRSSQSLLHSNGYNYLDWYLQKPGQSPQLLIYLGSNRASGVPDRFSGSGSGTHLTLKISRVEAEDVGVYYCMQTLQTPLTFGGGTKVEIKRTVAAPSVFIFPPSDEQLKSGTASVVCLLNNFYPREAKVQWKVDNALQSGNSQESVTEQDSKDSTYSLSSTLTLSKADYEKHKVYACEVTHQGLSSPVTKSFNRGEC

SEQ ID NO: 28 - protein, 475 aa, Homo sapiens
MDMRVPAQLLGLLLLWLRGARCEVQLVESGGGLVQPGGSLRLSCAASGFTFSNYWMSWVRQAPGKGLEWVASIKQDGSEKYYVDSVKGRFAISRDNAKNSLFLQMNSLRAEDTAVYYCARDLVLMVYDIDYYYYGMDVWGQGTTVTVSSASTKGPSVFPLAPCSRSTSESTAALGCLVKDYFPEPVTVSWNSGALTSGVHTFPAVLQSSGLYSLSSVVTVPSSNFGTQTYTCNVDHKPSNTKVDKTVERKCCVECPPCPAPPVAGPSVFLFPPKPKDTLMISRTPEVTCVVVDVSHEDPEVQFNWYVDGVEVHNAKTKPREEQFNSTFRVVSVLTVVHQDWLNGKEYKCKVSNKGLPAPIEKTISKTKGQPREPQVYTLPPSREEMTKNQVSLTCLVKGFYPSDIAVEWESNGQPENNYKTTPPMLDSDGSFFLYSKLTVDKSRWQQGNVFSCSVMHEALHNHYTQKSLSLSPGK

SEQ ID NO: 29 - protein, 235 aa, Homo sapiens
MTCSPLLLTLLIHCTGSWAQSVLTQPPSVSAAPGQKVTISCSGSSSNIGNNYVSWYQQLPGTAPKLLIYDNNKRPSGIPDRFSGSKSGTSTTLGITGLQTGDEADYYCGTWDSRLSAVVFGGGTKLTVLGQPKANPTVTLFPPSSEELQANKATLVCLISDFYPGAVTVAWKADGSPVKAGVETTKPSKQSNNKYAASSYLSLTPEQWKSHRSYSCQVTHEGSTVEKTVAPTECS

SEQ ID NO: 30 - protein, 475 aa, Homo sapiens
MEFGLSWVFLVALLRGVQCQVQLVESGGGVVQPGRSLRLSCAASGFTFSSFGMHWVRQAPGKGLEWVAVISFDGSIKYSVDSVKGRFTISRDNSKNTLFLQMNSLRAEDTAVYYCARDRLNYYDSSGYYHYKYYGMAVWGQGTTVTVSSASTKGPSVFPLAPCSRSTSESTAALGCLVKDYFPEPVTVSWNSGALTSGVHTFPAVLQSSGLYSLSSVVTVPSSNFGTQTYTCNVDHKPSNTKVDKTVERKCCVECPPCPAPPVAGPSVFLFPPKPKDTLMISRTPEVTCVVVDVSHEDPEVQFNWYVDGVEVHNAKTKPREEQFNSTFRVVSVLTVVHQDWLNGKEYKCKVSNKGLPAPIEKTISKTKGQPREPQVYTLPPSREEMTKNQVSLTCLVKGFYPSDIAVEWESNGQPENNYKTTPPMLDSDGSFFLYSKLTVDKSRWQQGNVFSCSVMHEALHNHYTQKSLSLSPGK

SEQ ID NO: 31 - protein, 234 aa, Homo sapiens
MDMRVPAQLLGLLLLWLRGARCYELTQPPSVSVSPGQTATITCSGDKLGERYASWYQQRPGQSPVLVIYQDIKRPSGIPERFSGSNSGNTATLTISGTQAMDEADYFCQAWYSSTNVLFGGGTKLTVLGQPKAAPSVTLFPPSSEELQANKATLVCLISDFYPGAVTVAWKADSSPVKAGVETTTPSKQSNNKYAASSYLSLTPEQWKSHRSYSCQVTHEGSTVEKTVAPTECS

SEQ ID NO: 32 - protein, 466 aa, Homo sapiens
MEFGLSWVFLVALLRGVQCQVQLVESGGGVVQPGRSLRLSCAASGFTFSSYGMHWVRQAPGKGLEWVAVIWYAESNKYYADSVKGRFTISRDNSKNTLYLQMNSLRAEDTAVYYCARAQEGIAPDAFDIWGQGTMVTVSSASTKGPSVFPLAPCSRSTSESTAALGCLVKDYFPEPVTVSWNSGALTSGVHTFPAVLQSSGLYSLSSVVTVPSSNFGTQTYTCNVDHKPSNTKVDKTVERKCCVECPPCPAPPVAGPSVFLFPPKPKDTLMISRTPEVTCVVVDVSHEDPEVQFNWYVDGVEVHNAKTKPREEQFNSTFRVVSVLTVVHQDWLNGKEYKCKVSNKGLPAPIEKTISKTKGQPREPQVYTLPPSREEMTKNQVSLTCLVKGFYPSDIAVEWESNGQPENNYKTTPPMLDSDGSFFLYSKLTVDKSRWQQGNVFSCSVMHEALHNHYTQKSLSLSPGK

SEQ ID NO: 33 - protein, 234 aa, Homo sapiens
MGSTAILGLLLAVLQGGRAEIVLTQSPGTLSLSPGERATLSCRASQSVSSSYLAWHQQKPGQAPRLLIYGASSRATGIPDRFSGSGSGTDFTLTISRLEPEDFAVYYCQQYGSSPWTFGQGTKVEIKRTVAAPSVFIFPPSDEQLKSGTASVVCLLNNFYPREAKVQWKVDNALQSGNSQESVTEQDSKDSTYSLSSTLTLSKADYEKHKVYACEVTHQGLSSPVTKSFNRGEC

SEQ ID NO: 34 - protein, 463 aa, Homo sapiens
MGSTAILGLLLAVLQGGRAEVQLLESGGGLVQPGGSLRLSCAASGFTFSTYVMSWVRQAPGKGLEWVSSISGSGLGSYYADSVKGRFTISRDNSKNTLYLQMNSLRAEDTAVYYCAKEAHRGPFDYWGQGTLVTVSSASTKGPSVFPLAPCSRSTSESTAALGCLVKDYFPEPVTVSWNSGALTSGVHTFPAVLQSSGLYSLSSVVTVPSSNFGTQTYTCNVDHKPSNTKVDKTVERKCCVECPPCPAPPVAGPSVFLFPPKPKDTLMISRTPEVTCVVVDVSHEDPEVQFNWYVDGVEVHNAKTKPREEQFNSTFRVVSVLTVVHQDWLNGKEYKCKVSNKGLPAPIEKTISKTKGQPREPQVYTLPPSREEMTKNQVSLTCLVKGFYPSDIAVEWESNGQPENNYKTTPPMLDSDGSFFLYSKLTVDKSRWQQGNVFSCSVMHEALHNHYTQKSLSLSPGK

SEQ ID NO: 35 - protein, 239 aa, Homo sapiens
MRLLAQLLGLLMLWVPGSSGDIVMTQTPLSSPVTLGQPASISCRSSQSLVHSDGNTYLSWLQQRPGQPPRLLIYKKFNRFSGVPDRFSGSGAGTDFTLKISRVEAEDVGVYYCMQATQIPLTFGPGTKVDIKRTVAAPSVFIFPPSDEQLKSGTASVVCLLNNFYPREAKVQWKVDNALQSGNSQESVTEQDSKDSTYSLSSTLTLSKADYEKHKVYACEVTHQGLSSPVTKSFNRGEC

SEQ ID NO: 36 - protein, 472 aa, Homo sapiens
MEFGLSWVFLVALLRGVQCQVQLVESGGGVVQPGRSLRLSCAASGFTFSFYGMHWVRQAPGKGLEWVAVIWYDGSNKYYADSVKGRFTISRDNSKNTLYLQMNSLRAEDTAVYYCARGGYDYVWGSYRRNSDFDYWGQGTLVTVSSASTKGPSVFPLAPCSRSTSESTAALGCLVKDYFPEPVTVSWNSGALTSGVHTFPAVLQSSGLYSLSSVVTVPSSNFGTQTYTCNVDHKPSNTKVDKTVERKCCVECPPCPAPPVAGPSVFLFPPKPKDTLMISRTPEVTCVVVDVSHEDPEVQFNWYVDGVEVHNAKTKPREEQFNSTFRVVSVLTVVHQDWLNGKEYKCKVSNKGLPAPIEKTISKTKGQPREPQVYTLPPSREEMTKNQVSLTCLVKGFYPSDIAVEWESNGQPENNYKTTPPMLDSDGSFFLYSKLTVDKSRWQQGNVFSCSVMHEALHNHYTQKSLSLSPGK

SEQ ID NO: 37 - protein, 235 aa, Homo sapiens
MEAPAQLLFLLLLWLPDTTGEIVMTQSPATLSVSPGERATLSCRASQSVDSNLAWYRQKPGQAPRLLIYGASTRATGIPARFSGSGSGTEFTLTISSLQSEDFAVYYCQQYINWPPITFGQGTRLEIKRTVAAPSVFIFPPSDEQLKSGTASVVCLLNNFYPREAKVQWKVDNALQSGNSQESVTEQDSKDSTYSLSSTLTLSKADYEKHKVYACEVTHQGLSSPVTKSFNRGEC

SEQ ID NO: 38 - protein, 465 aa, Homo sapiens
MKHLWFFLLLVAAPRWVLSQVQLQESGPGLVKPSETLSLTCTVSGGSISIYYWSWIRQPPGKGLEWIGYVYYSGSTNYNPSLKSRVTISVDTSKNQFSLKLNSVTAADTAVYYCARGGYDFWSGYFDYWGQGTLVTVSSASTKGPSVFPLAPCSRSTSESTAALGCLVKDYFPEPVTVSWNSGALTSGVHTFPAVLQSSGLYSLSSVVTVPSSNFGTQTYTCNVDHKPSNTKVDKTVERKCCVECPPCPAPPVAGPSVFLFPPKPKDTLMISRTPEVTCVVVDVSHEDPEVQFNWYVDGVEVHNAKTKPREEQFNSTFRVVSVLTVVHQDWLNGKEYKCKVSNKGLPAPIEKTISKTKGQPREPQVYTLPPSREEMTKNQVSLTCLVKGFYPSDIAVEWESNGQPENNYKTTPPMLDSDGSFFLYSKLTVDKSRWQQGNVFSCSVMHEALHNHYTQKSLSLSPGK

SEQ ID NO: 39 - protein, 240 aa, Homo sapiens
MVLQTQVFISLLLWISGAYGDIVLTQSPDSLAVSLGERATINCKSSQSILYSSSNENFLTWYQQKPGQPPKLLIYWASTRESGVPDRFSGSGSGTDFTLTISSLQPEDVAVYYCQQYFSVFRTFGQGTRVEIKRTVAAPSVFIFPPSDEQLKSGTASVVCLLNNFYPREAKVQWKVDNALQSGNSQESVTEQDSKDSTYSLSSTLTLSKADYEKHKVYACEVTHQGLSSPVTKSFNRGEC

SEQ ID NO: 40 - protein, 465 aa, Homo sapiens
MDWTWRILFLVAAATGAHSQVQLVQSGAEVKKPGASVKVSCKASGYTFTGYYIHWVRQAPGQGLEWMGWINPNSGGTNSAQKFRGRVTMTRDTSISTAYMELSRLRSDDTAVYYCAREGGYSYGYFDYWGQGTLVTVSSASTKGPSVFPLAPCSRSTSESTAALGCLVKDYFPEPVTVSWNSGALTSGVHTFPAVLQSSGLYSLSSVVTVPSSNFGTQTYTCNVDHKPSNTKVDKTVERKCCVECPPCPAPPVAGPSVFLFPPKPKDTLMISRTPEVTCVVVDVSHEDPEVQFNWYVDGVEVHNAKTKPREEQFNSTFRVVSVLTVVHQDWLNGKEYKCKVSNKGLPAPIEKTISKTKGQPREPQVYTLPPSREEMTKNQVSLTCLVKGFYPSDIAVEWESNGQPENNYKTTPPMLDSDGSFFLYSKLTVDKSRWQQGNVFSCSVMHEALHNHYTQKSLSLSPGK

SEQ ID NO: 41 - protein, 236 aa, Homo sapiens
MDMRVPAQLLGLLLLWFPGARCDIQMTQSPSSLSASVGDRVTITCRASQGIRNDLGWYQQKPGKAPKRLIYAASSLQSGVPSRFSGSGSGTEFTLTISSVQPEDFVTYYCLQHNSNPLTFGGGTKVEIKRTVAAPSVFIFPPSDEQLKSGTASVVCLLNNFYPREAKVQWKVDNALQSGNSQESVTEQDSKDSTYSLSSTLTLSKADYEKHKVYACEVTHQGLSSPVTKSFNRGEC

SEQ ID NO: 42 - protein, 473 aa, Homo sapiens
MEFGLSWVFLVALLRGVQCQVQLVESGGGVVQPGRSLRLSCAASGFTFSSYGMHWVRQAPGKGLEWVAVMWYDGSNKDYVDSVKGRFTISRDNSKNTLYLQMNRLRAEDTAVYYCAREKDHYDILTGYNYYYGLDVWGQGTTVTVSSASTKGPSVFPLAPCSRSTSESTAALGCLVKDYFPEPVTVSWNSGALTSGVHTFPAVLQSSGLYSLSSVVTVPSSNFGTQTYTCNVDHKPSNTKVDKTVERKCCVECPPCPAPPVAGPSVFLFPPKPKDTLMISRTPEVTCVVVDVSHEDPEVQFNWYVDGVEVHNAKTKPREEQFNSTFRVVSVLTVVHQDWLNGKEYKCKVSNKGLPAPIEKTISKTKGQPREPQVYTLPPSREEMTKNQVSLTCLVKGFYPSDIAVEWESNGQPENNYKTTPPMLDSDGSFFLYSKLTVDKSRWQQGNVFSCSVMHEALHNHYTQKSLSLSPGK

SEQ ID NO: 43 - protein, 235 aa, Homo sapiens
METPAQLLFLLLLWLPDTTGEIVLTQSPGTLSLSPGERATLSCRASQYISNTYLAWFQQKPGQAPRLLIYGAATRATGIPDRFSGSGSGTDFTFTISRLEPEDFAVYYCQQYGSSPWTFGQGTTVEIKRTVAAPSVFIFPPSDEQLKSGTASVVCLLNNFYPREAKVQWKVDNALQSGNSQESVTEQDSKDSTYSLSSTLTLSKADYEKHKVYACEVTHQGLSSPVTKSFNRGEC

SEQ ID NO: 44 - protein, 463 aa, Homo sapiens
MDWTWRILFLVAAATGAHSQVQLVQSGAEVKKPGASVKVSCKASGYTFTGYYMHWVRQAPGQGLEWMGWINPNSGGTNYAQRFRGRVTMTRDTSISTAYMELSRLRSDDTAVYYCARAPYDWTFDYWGQGTLVTVSSASTKGPSVFPLAPCSRSTSESTAALGCLVKDYFPEPVTVSWNSGALTSGVHTFPAVLQSSGLYSLSSVVTVPSSNFGTQTYTCNVDHKPSNTKVDKTVERKCCVECPPCPAPPVAGPSVFLFPPKPKDTLMISRTPEVTCVVVDVSHEDPEVQFNWYVDGVEVHNAKTKPREEQFNSTFRVVSVLTVVHQDWLNGKEYKCKVSNKGLPAPIEKTISKTKGQPREPQVYTLPPSREEMTKNQVSLTCLVKGFYPSDIAVEWESNGQPENNYKTTPPMLDSDGSFFLYSKLTVDKSRWQQGNVFSCSVMHEALHNHYTQKSLSLSPGK

SEQ ID NO: 45 - protein, 236 aa, Homo sapiens
MDMRVPAQLLGLLLLWLRGARCDIQMTQSPSSVSASVGDRVTITCRASQGISNWLAWYQQKPGTAPKLLIYAASSLQSGVPSRFSGSGSGTDFTLTISSLQPEDFATYYCQQANSFPFTFGPGTKVDIKRTVAAPSVFIFPPSDEQLKSGTASVVCLLNNFYPREAKVQWKVDNALQSGNSQESVTEQDSKDSTYSLSSTLTLSKADYEKHKVYACEVTHQGLSSPVTKSFNRGEC

SEQ ID NO: 46 - protein, 469 aa, Homo sapiens
MDMRVPAQLLGLLLLWLRGARCQVQLVQSGTEVKKPGASMKVSCKASGYTFTSYYMHWVRQAPGQGLEWMGIINPSGDSTSYAQKFQGRVTMTRDTSTNTVYMELSSLRSEDTAMYYCARDVEVRGISHFDYWGQGTLVTVSSASTKGPSVFPLAPCSRSTSESTAALGCLVKDYFPEPVTVSWNSGALTSGVHTFPAVLQSSGLYSLSSVVTVPSSNFGTQTYTCNVDHKPSNTKVDKTVERKCCVECPPCPAPPVAGPSVFLFPPKPKDTLMISRTPEVTCVVVDVSHEDPEVQFNWYVDGVEVHNAKTKPREEQFNSTFRVVSVLTVVHQDWLNGKEYKCKVSNKGLPAPIEKTISKTKGQPREPQVYTLPPSREEMTKNQVSLTCLVKGFYPSDIAVEWESNGQPENNYKTTPPMLDSDGSFFLYSKLTVDKSRWQQGNVFSCSVMHEALHNHYTQKSLSLSPGK

SEQ ID NO: 47 - protein, 238 aa, Homo sapiens
MGWSCIILFLVATATGVHSDIQLTQSPSSLSASVGDRVTMSCKSSQSVLYSANHKNYLAWYQQKPGKAPKLLIYWASTRESGVPSRFSGSGSGTDFTFTISSLQPEDIATYYCHQYLSSWTFGGGTKVQIKRTVAAPSVFIFPPSDEQLKSGTASVVCLLNNFYPREAKVQWKVDNALQSGNSQESVTEQDSKDSTYSLSSTLTLSKADYEKHKVYACEVTHQGLSSPVTKSFNRGEC

SEQ ID NO: 48 - protein, 465 aa, Homo sapiens
MGWSCIILFLVATATGVHSQVQLVQSGAEVKKPGSSVKVSCKASGYTFTSYWLHWVRQAPGQGLEWIGYINPRNDYTEYNQNFKDKATITADESTNTAYMELSSLRSEDTAFYFCARRDITTFYWGQGTTVTVSSASTKGPSVFPLAPSSKSTSGGTAALGCLVKDYFPEPVTVSWNSGALTSGVHTFPAVLQSSGLYSLSSVVTVPSSSLGTQTYICNVNHKPSNTKVDKRVEPKSCDKTHTCPPCPAPELLGGPSVFLFPPKPKDTLMISRTPEVTCVVVDVSHEDPEVKFNWYVDGVEVHNAKTKPREEQYNSTYRVVSVLTVLHQDWLNGKEYKCKVSNKALPAPIEKTISKAKGQPREPQVYTLPPSREEMTKNQVSLTCLVKGFYPSDIAVEWESNGQPENNYKTTPPVLDSDGSFFLYSKLTVDKSRWQQGNVFSCSVMHEALHNHYTQKSLSLSPGK

SEQ ID NO: 49 - protein, 235 aa, Homo sapiens
METPAQLLFLLLLWLPDTTGEIVLTQSPGTLSLSPGERATLSCRASQSVSSSYLAWYQQKPGQAPRLLIYGASSRATGIPDRFSGSGSGTDFTLTISRLEPEDFAVYYCQRSGGSSFTFGPGTKVDIKRTVAAPSVFIFPPSDEQLKSGTASVVCLLNNFYPREAKVQWKVDNALQSGNSQESVTEQDSKDSTYSLSSTLTLSKADYEKHKVYACEVTHQGLSSPVTKSFNRGEC

SEQ ID NO: 50 - protein, 466 aa, Homo sapiens
MGSTAILALLLAVLQGVCAEVQLVQSGAEVKKPGESLKISCKGSGYNFTSYWIGWVRQMPGKGLELMGIIYPGDSDTRYSPSFQGQVTISADKSISTAYLQWSSLKASDTAMYYCGSGSYFYFDLWGRGTLVTVSSASTKGPSVFPLAPSSKSTSGGTAALGCLVKDYFPEPVTVSWNSGALTSGVHTFPAVLQSSGLYSLSSVVTVPSSSLGTQTYICNVNHKPSNTKVDKKVEPKSCDKTHTCPPCPAPELLGGPSVFLFPPKPKDTLMISRTPEVTCVVVDVSHEDPEVKFNWYVDGVEVHNAKTKPREEQYNSTYRVVSVLTVLHQDWLNGKEYKCKVSNKALPAPIEKTISKAKGQPREPQVYTLPPSRDELTKNQVSLTCLVKGFYPSDIAVEWESNGQPENNYKTTPPVLDSDGSFFLYSKLTVDKSRWQQGNVFSCSVMHEALHNHYTQKSLSLSPGK

SEQ ID NO: 51 - protein, 241 aa, Homo sapiens
MDMRVPAQLLGLLLLWLRGARCDIVMTQSPLSLPVTPGEPASISCRSSQSLLHSHGYNYLDWYLQKPGQSPQLLIYLGSNRASGVPDRFSGSGSGTDFTLKISRVEAEDVGVYYCMQGTHWPPTFGQGTKLEIKRTVAAPSVFIFPPSDEQLKSGTASVVCLLNNFYPREAKVQWKVDNALQSGNSQESVTEQDSKDSTYSLSSTLTLSKADYEKHKVYACEVTHQGLSSPVTKSFNRGEC

SEQ ID NO: 52 - protein, 470 aa, Homo sapiens
MDMRVPAQLLGLLLLWLRGARCEVQLVQSGGGVVQPGRSLRLSCAASGFTFSSYGMHWVRQAPGKGLEWVSYISSSGSTIYYADSVKGRFTISRDNAKNSLYLQMNSLRAEDTAVYYCARDLLDYDLLTGYGYWGQGTLVTVSSASTKGPSVFPLAPCSRSTSESTAALGCLVKDYFPEPVTVSWNSGALTSGVHTFPAVLQSSGLYSLSSVVTVPSSNFGTQTYTCNVDHKPSNTKVDKTVERKCCVECPPCPAPPVAGPSVFLFPPKPKDTLMISRTPEVTCVVVDVSHEDPEVQFNWYVDGVEVHNAKTKPREEQFNSTFRVVSVLTVVHQDWLNGKEYKCKVSNKGLPAPIEKTISKTKGQPREPQVYTLPPSREEMTKNQVSLTCLVKGFYPSDIAVEWESNGQPENNYKTTPPMLDSDGSFFLYSKLTVDKSRWQQGNVFSCSVMHEALHNHYTQKSLSLSPGK

SEQ ID NO: 53 - protein, 235 aa, Homo sapiens
METPAQLLFLLLLWLPDTTGEIVLTQSPGTLSLSPGERATLSCRASQGISRSYLAWYQQKPGQAPSLLIYGASSRATGIPDRFSGSGSGTDFTLTISRLEPEDFAVYYCQQFGSSPWTFGQGTKVEIKRTVAAPSVFIFPPSDEQLKSGTASVVCLLNNFYPREAKVQWKVDNALQSGNSQESVTEQDSKDSTYSLSSTLTLSKADYEKHKVYACEVTHQGLSSPVTKSFNRGEC

SEQ ID NO: 54 - protein, 471 aa, Homo sapiens
MKHLWFFLLLVAAPRWVLSQVQLQESGPGLVKPSQTLSLTCTVSGGSISSGDYFWSWIRQLPGKGLEWIGHIHNSGTTYYNPSLKSRVTISVDTSKKQFSLRLSSVTAADTAVYYCARDRGGDYYYGMDVWGQGTTVTVSSASTKGPSVFPLAPSSKSTSGGTAALGCLVKDYFPEPVTVSWNSGALTSGVHTFPAVLQSSGLYSLSSVVTVPSSSLGTQTYICNVNHKPSNTKVDKRVEPKSCDKTHTCPPCPAPELLGGPSVFLFPPKPKDTLMISRTPEVTCVVVDVSHEDPEVKFNWYVDGVEVHNAKTKPREEQYNSTYRVVSVLTVLHQDWLNGKEYKCKVSNKALPAPIEKTISKAKGQPREPQVYTLPPSREEMTKNQVSLTCLVKGFYPSDIAVEWESNGQPENNYKTTPPVLDSDGSFFLYSKLTVDKSRWQQGNVFSCSVMHEALHNHYTQKSLSLSPGK

SEQ ID NO: 55 - protein, 236 aa, Homo sapiens
MDMRVPAQLLGLLLLWLSGARCDIQMTQSPSSLSASVGDRVTITCQASQDISNYLNWYQQKPGKAPKLLIYDASNLETGVPSRFSGSGSGTDFTFTISSLQPEDIATYFCQHFDHLPLAFGGGTKVEIKRTVAAPSVFIFPPSDEQLKSGTASVVCLLNNFYPREAKVQWKVDNALQSGNSQESVTEQDSKDSTYSLSSTLTLSKADYEKHKVYACEVTHQGLSSPVTKSFNRGEC

SEQ ID NO: 56 - protein, 464 aa, Homo sapiens
MKHLWFFLLLVAAPRWVLSQVQLQESGPGLVKPSETLSLTCTVSGGSVSSGDYYWTWIRQSPGKGLEWIGHIYYSGNTNYNPSLKSRLTISIDTSKTQFSLKLSSVTAADTAIYYCVRDRVTGAFDIWGQGTMVTVSSASTKGPSVFPLAPCSRSTSESTAALGCLVKDYFPEPVTVSWNSGALTSGVHTFPAVLQSSGLYSLSSVVTVPSSNFGTQTYTCNVDHKPSNTKVDKTVERKCCVECPPCPAPPVAGPSVFLFPPKPKDTLMISRTPEVTCVVVDVSHEDPEVQFNWYVDGVEVHNAKTKPREEQFNSTFRVVSVLTVVHQDWLNGKEYKCKVSNKGLPAPIEKTISKTKGQPREPQVYTLPPSREEMTKNQVSLTCLVKGFYPSDIAVEWESNGQPENNYKTTPPMLDSDGSFFLYSKLTVDKSRWQQGNVFSCSVMHEALHNHYTQKSLSLSPGK

SEQ ID NO: 57 - protein, 236 aa, Homo sapiens
METPAQLLFLLLLWLPDTASEIVLTQSPGTLSLSPGERATLSCRASQSVSNSYLAWYQQKPGQAPRLLIYGASSRAPGIPDRFSGSGSGTDFTLTISRLEPEDFAVYYCQQYDHSAGWTFGQGTKVEIKRTVAAPSVFIFPPSDEQLKSGTASVVCLLNNFYPREAKVQWKVDNALQSGNSQESVTEQDSKDSTYSLSSTLTLSKADYEKHKVYACEVTHQGLSSPVTKSFNRGEC

SEQ ID NO: 58 - protein, 460 aa, Homo sapiens
MGSTAILGLLLAVLQGVASEVQLVESGGGLVQPGGSLRLSCAASGFTFSRNAMFWVRQAPGKGLEWVSGIGTGGATSYADSVKGRFTISRDNAKNSLYLQMNSLRAEDTAVYYCARGRYYFPWWGQGTLVTVSSASTKGPSVFPLAPCSRSTSESTAALGCLVKDYFPEPVTVSWNSGALTSGVHTFPAVLQSSGLYSLSSVVTVPSSNFGTQTYTCNVDHKPSNTKVDKTVERKCCVECPPCPAPPVAGPSVFLFPPKPKDTLMISRTPEVTCVVVDVSHEDPEVQFNWYVDGVEVHNAKTKPREEQFNSTFRVVSVLTVVHQDWLNGKEYKCKVSNKGLPAPIEKTISKTKGQPREPQVYTLPPSREEMTKNQVSLTCLVKGFYPSDIAVEWESNGQPENNYKTTPPMLDSDGSFFLYSKLTVDKSRWQQGNVFSCSVMHEALHNHYTQKSLSLSPGK

SEQ ID NO: 59 - protein, 234 aa, Homo sapiens
METPAQLLFLLLLWLPDTTGEIVLTQSPGTLSLSPGERATLSCRASQSVSSSYLAWYQQKPGQAPRLLIYGASRRATGIPDRFSGSGSGTDFTLTISRLEPEDFAVYYCQRYGSSHTFGQGTKLEISRTVAAPSVFIFPPSDEQLKSGTASVVCLLNNFYPREAKVQWKVDNALQSGNSQESVTEQDSKDSTYSLSSTLTLSKADYEKHKVYACEVTHQGLSSPVTKSFNRGEC

SEQ ID NO: 60 - protein, 467 aa, Homo sapiens
MGSTAILALLLAVLQGVCAEVQLVQSGAEVKKPGESLKISCKVSGYFFTTYWIGWVRQMPGKGLEYMGIIYPGDSDTRYSPSFQGQVTISADKSISTAYLQWSSLKASDTAMYYCARGGNWNCFDYWGQGTLVTVSSASTKGPSVFPLAPSSKSTSGGTAALGCLVKDYFPEPVTVSWNSGALTSGVHTFPAVLQSSGLYSLSSVVTVPSSSLGTQTYICNVNHKPSNTKVDKRVEPKSCDKTHTCPPCPAPELLGGPSVFLFPPKPKDTLMISRTPEVTCVVVDVSHEDPEVKFNWYVDGVEVHNAKTKPREEQYNSTYRVVSVLTVLHQDWLNGKEYKCKVSNKALPAPIEKTISKAKGQPREPQVYTLPPSRDELTKNQVSLTCLVKGFYPSDIAVEWESNGQPENNYKTTPPVLDSDGSFFLYSKLTVDKSRWQQGNVFSCSVMHEALHNHYTQKSLSLSPGK

SEQ ID NO: 61 - protein, 241 aa, Homo sapiens
MDMRVPAQLLGLLLLWLRGARCDVVMTQSPLSLPVTPGEPASISCRSSQSLLHSNGYNYLDWYLQKPGQSPQLLIYLGSNRASGVPDRFSGSGSGTDFTLKISRVEAEDVGVYYCMQGTHWPLTFGQGTKVEIKRTVAAPSVFIFPPSDEQLKSGTASVVCLLNNFYPREAKVQWKVDNALQSGNSQESVTEQDSKDSTYSLSSTLTLSKADYEKHKVYACEVTHQGLSSPVTKSFNRGEC

SEQ ID NO: 62 - protein, 471 aa, Homo sapiens
MDMRVPAQLLGLLLLWLRGARCQVQLQESGPGLVKPSGTLSLTCAVSGGSISSSNWWSWVRQPPGKGLEWIGEIYHSGSTNYNPSLKSRVTISVDKSKNQFSLKLSSVTAADTAVYYCARWTGRTDAFDIWGQGTMVTVSSASTKGPSVFPLAPSSKSTSGGTAALGCLVKDYFPEPVTVSWNSGALTSGVHTFPAVLQSSGLYSLSSVVTVPSSSLGTQTYICNVNHKPSNTKVDKKVEPKSCDKTHTCPPCPAPELLGGPSVFLFPPKPKDTLMISRTPEVTCVVVDVSHEDPEVKFNWYVDGVEVHNAKTKPREEQYNSTYRVVSVLTVLHQDWLNGKEYKCKVSNKALPAPIEKTISKAKGQPREPQVYTLPPSRDELTKNQVSLTCLVKGFYPSDIAVEWESNGQPENNYKTTPPVLDSDGSFFLYSKLTVDKSRWQQGNVFSCSVMHEALHNHYTQKSLSLSPGK

SEQ ID NO: 63 - protein, 234 aa, Homo sapiens
MEAPAQLLFLLLLWLPDTTGEIVMTQSPATLSVSPGERATLSCRASQSVSSNLAWFQQKPGQAPRPLIYDASTRATGVPARFSGSGSGTDFTLTISSLQSEDFAVYYCQQYDNWPLTFGGGTKVEIKRTVAAPSVFIFPPSDEQLKSGTASVVCLLNNFYPREAKVQWKVDNALQSGNSQESVTEQDSKDSTYSLSSTLTLSKADYEKHKVYACEVTHQGLSSPVTKSFNRGEC

SEQ ID NO: 64 - protein, 461 aa, Homo sapiens
MEWTWRVLFLVAAATGAHSQVQLVQSGAEVKKPGASVKVSCKASGYTFTRYGISWVRQAPGQGLEWMGWISTYSGNTNYAQKLQGRVTMTTDTSTSTAYMELRSLRSDDTAVYYCARRQLYFDYWGQGTLVTVSSASTKGPSVFPLAPCSRSTSESTAALGCLVKDYFPEPVTVSWNSGALTSGVHTFPAVLQSSGLYSLSSVVTVPSSNFGTQTYTCNVDHKPSNTKVDKTVERKCCVECPPCPAPPVAGPSVFLFPPKPKDTLMISRTPEVTCVVVDVSHEDPEVQFNWYVDGVEVHNAKTKPREEQFNSTFRVVSVLTVVHQDWLNGKEYKCKVSNKGLPAPIEKTISKTKGQPREPQVYTLPPSREEMTKNQVSLTCLVKGFYPSDIAVEWESNGQPENNYKTTPPMLDSDGSFFLYSKLTVDKSRWQQGNVFSCSVMHEALHNHYTQKSLSLSPGK

SEQ ID NO: 65 - protein, 239 aa, Homo sapiens
MRLPAQLLGLLMLWIPGSSADIVMTQTPLSLSVTPGQPASISCKSGQSLLHSDGKTYLYWYLQKPGQPPQFLIYEVSNRFSRVPDRFSGSGSGTDFTLRISRVEAEDVGIYYCMQSIQLPWTFGQGTQVEIKRTVAAPSVFIFPPSDEQLKSGTASVVCLLNNFYPREAKVQWKVDNALQSGNSQESVTEQDSKDSTYSLSSTLTLSKADYEKHKVYACEVTHQGLSSPVTKSFNRGEC

SEQ ID NO: 66 - protein, 459 aa, Homo sapiens
MEFGLSWVFLVALLRGVQCQVQLVESGGGVVQPGRSLRLSCAASGFTFSGYGMHWVRQAPGKGLEWVAVISYDGNDKYYADSVKGRFTISRDNAKNTLYLQMNSLRAEDTAVYYCARELRVLWGQGTLVTVSSASTKGPSVFPLAPCSRSTSESTAALGCLVKDYFPEPVTVSWNSGALTSGVHTFPAVLQSSGLYSLSSVVTVPSSNFGTQTYTCNVDHKPSNTKVDKTVERKCCVECPPCPAPPVAGPSVFLFPPKPKDTLMISRTPEVTCVVVDVSHEDPEVQFNWYVDGVEVHNAKTKPREEQFNSTFRVVSVLTVVHQDWLNGKEYKCKVSNKGLPAPIEKTISKTKGQPREPQVYTLPPSREEMTKNQVSLTCLVKGFYPSDIAVEWESNGQPENNYKTTPPMLDSDGSFFLYSKLTVDKSRWQQGNVFSCSVMHEALHNHYTQKSLSLSPGK

SEQ ID NO: 67 - protein, 235 aa, Homo sapiens
MDMRVPAQLLGLLLLWLRGARCDIQMTQSPSSLSASVGDRVTITCRASQDISSYLNWYQQKPGKAPKLLIYSTSRLNSGVPSRFSGSGSGTDFTLTISSLQPEDFATYYCQQDIKHPTFGQGTKVEIKRTVAAPSVFIFPPSDEQLKSGTASVVCLLNNFYPREAKVQWKVDNALQSGNSQESVTEQDSKDSTYSLSSTLTLSKADYEKHKVYACEVTHQGLSSPVTKSFNRGEC

SEQ ID NO: 68 - protein, 465 aa, Homo sapiens
MDWTWRILFLVAAATGAHSEVQLVQSGAEVKKPGSSVKVSCKASGFTFTDYIMHWVRQAPGQGLEWMGYINPYNDDTEYNEKFKGRVTITADKSTSTAYMELSSLRSEDTAVYYCARSIYYYDAPFAYWGQGTLVTVSSASTKGPSVFPLAPCSRSTSESTAALGCLVKDYFPEPVTVSWNSGALTSGVHTFPAVLQSSGLYSLSSVVTVPSSNFGTQTYTCNVDHKPSNTKVDKTVERKCCVECPPCPAPPVAGPSVFLFPPKPKDTLMISRTPEVTCVVVDVSHEDPEVQFNWYVDGVEVHNAKTKPREEQFNSTFRVVSVLTVVHQDWLNGKEYKCKVSNKGLPAPIEKTISKTKGQPREPQVYTLPPSREEMTKNQVSLTCLVKGFYPSDIAVEWESNGQPENNYKTTPPMLDSDGSFFLYSKLTVDKSRWQQGNVFSCSVMHEALHNHYTQKSLSLSPGK

SEQ ID NO: 69 - protein, 233 aa, Homo sapiens
MGSTAILGLLLAVLQGGRASYVLTQPPSVSVAPGQTARITCGGNNLGSKSVHWYQQKPGQAPVLVVYDDSDRPSWIPERFSGSNSGNTATLTISRGEAGDEADYYCQVWDSSSDHVVFGGGTKLTVLGQPKAAPSVTLFPPSSEELQANKATLVCLISDFYPGAVTVAWKADSSPVKAGVETTTPSKQSNNKYAASSYLSLTPEQWKSHRSYSCQVTHEGSTVEKTVAPTECS

SEQ ID NO: 70 - protein, 467 aa, Homo sapiens
MGSTAILGLLLAVLQGGRAQMQLVESGGGVVQPGRSLRLSCAASGFTFRTYGMHWVRQAPGKGLEWVAVIWYDGSNKHYADSVKGRFTITRDNSKNTLNLQMNSLRAEDTAVYYCARAPQWELVHEAFDIWGQGTMVTVSSASTKGPSVFPLAPCSRSTSESTAALGCLVKDYFPEPVTVSWNSGALTSGVHTFPAVLQSSGLYSLSSVVTVPSSNFGTQTYTCNVDHKPSNTKVDKTVERKCCVECPPCPAPPVAGPSVFLFPPKPKDTLMISRTPEVTCVVVDVSHEDPEVQFNWYVDGVEVHNAKTKPREEQFNSTFRVVSVLTVVHQDWLNGKEYKCKVSNKGLPAPIEKTISKTKGQPREPQVYTLPPSREEMTKNQVSLTCLVKGFYPSDIAVEWESNGQPENNYKTTPPMLDSDGSFFLYSKLTVDKSRWQQGNVFSCSVMHEALHNHYTQKSLSLSPGK

SEQ ID NO: 71 - protein, 234 aa, Homo sapiens
MGVPTHLLGLLLLWITHAICDIRMTQSPASLSASLGETVNIECLASEDIYSDLAWYQQKPGKSPQLLIYNANSLQNGVPSRFSGSGSGTQYSLKINSLQSEDVATYFCQQYNNYPPTFGGGTKLELKRADAAPTVSIFPPSTEQLATGGASVVCLMNNFYPRDISVKWKIDGTERRDGVLDSVTDQDSKDSTYSMSSTLSLTKADYESHNLYTCEVVHKTSSSPVVKSFNRNEC

SEQ ID NO: 72 - protein, 465 aa, Homo sapiens
MDIRLSLAFLVLFIKGVQCEVQLVESGGGLVQPANSLKLSCAASGFTFSDYAMAWVRQSPKKGLEWVATIIYDGSSTYYRDSVKGRFTISRDNAKSTLYLQMDSLRSEDTATYYCATGLGIATDYFDYWGQGVLVTVSSAETTAPSVYPLAPGTALKSNSMVTLGCLVKGYFPEPVTVTWNSGALSSGVHTFPAVLQSGLYTLTSSVTVPSSTWPSQTVTCNVAHPASSTKVDKKIVPRNCGGDCKPCICTGSEVSSVFIFPPKPKDVLTITLTPKVTCVVVDISQDDPEVHFSWFVDDVEVHTAQTRPPEEQFNSTFRSVSELPILHQDWLNGRTFRCKVTSAAFPSPIEKTISKPEGRTQVPHVYTMSPTKEEMTQNEVSITCMVKGFYPPDIYVEWQMNGQPQENYKNTPPTMDTDGSYFLYSKLNVKKEKWQQGNTFTCSVLHEGLHNHHTEKSLSHSPGK

SEQ ID NO: 73 - protein, 237 aa, Homo sapiens
MDMRVPAQLLGLLLLWLRGARCESALTQPASVSGSPGQSITISCTGTSSDVGGYNSVSWYQQHPGKAPKLMIYEVSNRPSGVSNRFSGSKSGNTASLTISGLQAEDEADYYCNSYTSTSMVFGGGTKLTVLGQPKAAPSVTLFPPSSEELQANKATLVCLISDFYPGAVTVAWKADSSPVKAGVETTTPSKQSNNKYAASSYLSLTPEQWKSHRSYSCQVTHEGSTVEKTVAPTECS

SEQ ID NO: 74 - protein, 460 aa, Homo sapiens
MDWTWRILFLVAAATGVHSEVQLVQSGAEVKKPGASVKVSCKASGYTLTSYGISWVRQAPGQGLEWMGWVSFYNGNTNYAQKLQGRGTMTTDPSTSTAYMELRSLRSDDTAVYYCARGYGMDVWGQGTTVTVSSASTKGPSVFPLAPCSRSTSESTAALGCLVKDYFPEPVTVSWNSGALTSGVHTFPAVLQSSGLYSLSSVVTVPSSNFGTQTYTCNVDHKPSNTKVDKTVERKCCVECPPCPAPPVAGPSVFLFPPKPKDTLMISRTPEVTCVVVDVSHEDPEVQFNWYVDGVEVHNAKTKPREEQFNSTFRVVSVLTVVHQDWLNGKEYKCKVSNKGLPAPIEKTISKTKGQPREPQVYTLPPSREEMTKNQVSLTCLVKGFYPSDIAVEWESNGQPENNYKTTPPMLDSDGSFFLYSKLTVDKSRWQQGNVFSCSVMHEALHNHYTQKSLSLSPGK

SEQ ID NO: 75 - protein, 234 aa, Homo sapiens
METPAQLLFLLLLWLPDTTGEIVMTQSPATLSVSPGERATLSCRASQSVSSNLAWYQQKPGQAPRLLIYGAATRATGIPARVSGSGSGTEFTLTISSLQSEDFAVYYCQQYNNWPLTFGGGTKVEIKRTVAAPSVFIFPPSDEQLKSGTASVVCLLNNFYPREAKVQWKVDNALQSGNSQESVTEQDSKDSTYSLSSTLTLSKADYEKHKVYACEVTHQGLSSPVTKSFNRGEC

SEQ ID NO: 76 - protein, 472 aa, Homo sapiens
MDMRVPAQLLGLLLLWLRGARCQVQLVESGGGVVQPGRSLRLSCAASGFTFSNYGMHWVRQAPGEGLEWVAAIWFDASDKYYADAVKGRFTISRDNSKNTLYLQMNSLRAEDTAVYYCARDQAIFGVVPDYWGQGTLVTVSSASTKGPSVFPLAPSSKSTSGGTAALGCLVKDYFPEPVTVSWNSGALTSGVHTFPAVLQSSGLYSLSSVVTVPSSSLGTQTYICNVNHKPSNTKVDKKVEPKSCDKTHTCPPCPAPELLGGPSVFLFPPKPKDTLMISRTPEVTCVVVDVSHEDPEVKFNWYVDGVEVHNAKTKPCEEQYGSTYRCVSVLTVLHQDWLNGKEYKCKVSNKALPAPIEKTISKAKGQPREPQVYTLPPSREEMTKNQVSLTCLVKGFYPSDIAVEWESNGQPENNYKTTPPVLDSDGSFFLYSKLTVDKSRWQQGNVFSCSVMHEALHNHYTQKSLSLSPGK

SEQ ID NO: 77 - protein, 231 aa, Homo sapiens
MAWIPLFLGVLAYCTGSVASYEVTQAPSVSVSPGQTASITCSGDKLGDKYACWYQQKPGQSPVLVIYQDSKRPSGIPERFSGSNSGNTATLTISGTQAMDEADYYCQAWDSSTAVFGGGTKLTVLGQPKAAPSVTLFPPSSEELQANKATLVCLISDFYPGAVTVAWKADSSPVKAGVETTTPSKQSNNKYAASSYLSLTPEQWKSHRSYSCQVTHEGSTVEKTVAPTECS

SEQ ID NO: 78 - protein, 467 aa, Homo sapiens
MDWTWSILFLVAAATGAHSQVQLVQSGAEVKKPGASVKVSCKASGYTFTSYGLSWVRQAPGQGLEWMGWIIPYNGNTNSAQKLQGRVTMTTDTSTSTAYMELRSLRSDDTAVYFCARDRDYGVNYDAFDIWGQGTMVTVSSASTKGPSVFPLAPCSRSTSESTAALGCLVKDYFPEPVTVSWNSGALTSGVHTFPAVLQSSGLYSLSSVVTVPSSNFGTQTYTCNVDHKPSNTKVDKTVERKCCVECPPCPAPPVAGPSVFLFPPKPKDTLMISRTPEVTCVVVDVSHEDPEVQFNWYVDGVEVHNAKTKPREEQFNSTFRVVSVLTVVHQDWLNGKEYKCKVSNKGLPAPIEKTISKTKGQPREPQVYTLPPSREEMTKNQVSLTCLVKGFYPSDIAVEWESNGQPENNYKTTPPMLDSDGSFFLYSKLTVDKSRWQQGNVFSCSVMHEALHNHYTQKSLSLSPGK

SEQ ID NO: 79 - protein, 235 aa, Homo sapiens
MAWAPLLLTLLAHCTGSWANFMLTQPHSVSESPGKTVAISCTRNSGSIASNSVQWYQQRPGSSPTTVIFEDNQRPSGVPDRFSGSIDSSSNSASLTISGLKTEDEADYYCQSYDSNNWVFGGGTKLTVLGQPKANPTVTLFPPSSEELQANKATLVCLISDFYPGAVTVAWKADGSPVKAGVETTKPSKQSNNKYAASSYLSLTPEQWKSHRSYSCQVTHEGSTVEKTVAPTECS

SEQ ID NO: 80 - protein, 470 aa, Homo sapiens
MEFGLSWVFLVALLRGVQCQVQLVESGGGVVQPGRSLRLSCAASGFTFSSYVMHWVRQAPGKGLEWVAVIWYDGSNKYYADSVKGRFTISRDNSKNTLYLQMNSLRAEDTAVYYCAREGYDYGEDYYYYGMDVWGQGTTVTVSSASTKGPSVFPLAPCSRSTSESTAALGCLVKDYFPEPVTVSWNSGALTSGVHTFPAVLQSSGLYSLSSVVTVPSSNFGTQTYTCNVDHKPSNTKVDKTVERKCCVECPPCPAPPVAGPSVFLFPPKPKDTLMISRTPEVTCVVVDVSHEDPEVQFNWYVDGVEVHNAKTKPREEQFNSTFRVVSVLTVVHQDWLNGKEYKCKVSNKGLPAPIEKTISKTKGQPREPQVYTLPPSREEMTKNQVSLTCLVKGFYPSDIAVEWESNGQPENNYKTTPPMLDSDGSFFLYSKLTVDKSRWQQGNVFSCSVMHEALHNHYTQKSLSLSPGK

SEQ ID NO: 81 - protein, 236 aa, Homo sapiens
MDMRVPAQLLGLLLLWLRGARCDIQMTQSPSSLSASVGDRVTITCRASQDISNYLNWYQQKPGKAPKLLIYYTSRLLSGVPSRFSGSGSGTDFTLTISSLQPEDFATYYCQQGDTLPYTFGGGTKVEIKRTVAAPSVFIFPPSDEQLKSGTASVVCLLNNFYPREAKVQWKVDNALQSGNSQESVTEQDSKDSTYSLSSTLTLSKADYEKHKVYACEVTHQGLSSPVTKSFNRGEC

SEQ ID NO: 82 - protein, 468 aa, Homo sapiens
MDWTWRILFLVAAATGAHSEVQLVQSGAEVKKPGASVKVSCKASGYTFTDYNMHWVRQAPGQGLEWMGEINPNSGGAGYNQKFKGRVTMTTDTSTSTAYMELRSLRSDDTAVYYCARLGYDDIYDDWYFDVWGQGTTVTVSSASTKGPSVFPLAPCSRSTSESTAALGCLVKDYFPEPVTVSWNSGALTSGVHTFPAVLQSSGLYSLSSVVTVPSSNFGTQTYTCNVDHKPSNTKVDKTVERKCCVECPPCPAPPVAGPSVFLFPPKPKDTLMISRTPEVTCVVVDVSHEDPEVQFNWYVDGVEVHNAKTKPREEQFNSTFRVVSVLTVVHQDWLNGKEYKCKVSNKGLPAPIEKTISKTKGQPREPQVYTLPPSREEMTKNQVSLTCLVKGFYPSDIAVEWESNGQPENNYKTTPPMLDSDGSFFLYSKLTVDKSRWQQGNVFSCSVMHEALHNHYTQKSLSLSPGK

SEQ ID NO: 83 - protein, 240 aa, Homo sapiens
MVLQTQVFISLLLWISGAYGDIVMTQSPDSLAVSLGERATINCKSSQSVLDSSDNKNYLAWYQQKPGQPPKLLIYWASNRESGVPDRFSGSGSGTDFTLTISSLQAEDVAVYYCQQYYSDPFTFGPGTKVDIKRTVAAPSVFIFPPSDEQLKSGTASVVCLLNNFYPREAKVQWKVDNALQSGNSQESVTEQDSKDSTYSLSSTLTLSKADYEKHKVYACEVTHQGLSSPVTKSFNRGEC

SEQ ID NO: 84 - protein, 465 aa, Homo sapiens
MDWTWSILFLVAAPTGAHSQVQLVQSGAEVKKPGASVKVSCKASGYTFTSYGISWVRQAPGQGLEWMGWISAYNGNTNYAQKLQGRVTMTTDTSTSTAYMELRSLRSDDTAVYYCARESWFGEVFFDYWGQGTLVTVSSASTKGPSVFPLAPCSRSTSESTAALGCLVKDYFPEPVTVSWNSGALTSGVHTFPAVLQSSGLYSLSSVVTVPSSNFGTQTYTCNVDHKPSNTKVDKTVERKCCVECPPCPAPPVAGPSVFLFPPKPKDTLMISRTPEVTCVVVDVSHEDPEVQFNWYVDGVEVHNAKTKPREEQFNSTFRVVSVLTVVHQDWLNGKEYKCKVSNKGLPAPIEKTISKTKGQPREPQVYTLPPSREEMTKNQVSLTCLVKGFYPSDIAVEWESNGQPENNYKTTPPMLDSDGSFFLYSKLTVDKSRWQQGNVFSCSVMHEALHNHYTQKSLSLSPGK

SEQ ID NO: 85 - protein, 236 aa, Homo sapiens
MDMRVPAQLLGLLLLWLRGARCDIQMTQSPSSVSASVGDRVTITCRASQGISSWLAWYQQKPGKAPKLLIYGASNLESGVPSRFSGSGSGTDFTLTISSLQPEDFANYYCQQANSFPWTFGQGTKVEIKRTVAAPSVFIFPPSDEQLKSGTASVVCLLNNFYPREAKVQWKVDNALQSGNSQESVTEQDSKDSTYSLSSTLTLSKADYEKHKVYACEVTHQGLSSPVTKSFNRGEC

SEQ ID NO: 86 - protein, 466 aa, Homo sapiens
MDMRVPAQLLGLLLLWLRGARCQVQLVQSGAEVKKPGASVKVSCKVSGYTLSDLSIHWVRQAPGKGLEWMGGFDPQDGETIYAQKFQGRVTMTEDTSTDTAYMELSSLKSEDTAVYYCATGSSSSWFDPWGQGTLVTVSSASTKGPSVFPLAPCSRSTSESTAALGCLVKDYFPEPVTVSWNSGALTSGVHTFPAVLQSSGLYSLSSVVTVPSSNFGTQTYTCNVDHKPSNTKVDKTVERKCCVECPPCPAPPVAGPSVFLFPPKPKDTLMISRTPEVTCVVVDVSHEDPEVQFNWYVDGVEVHNAKTKPREEQFNSTFRVVSVLTVVHQDWLNGKEYKCKVSNKGLPAPIEKTISKTKGQPREPQVYTLPPSREEMTKNQVSLTCLVKGFYPSDIAVEWESNGQPENNYKTTPPMLDSDGSFFLYSKLTVDKSRWQQGNVFSCSVMHEALHNHYTQKSLSLSPGK